European Patent Specification EP 3 850 099 B1, published September 3, 2025. Title: microRNA inhibitors for use in treating metabolic diseases. Applicant: Helmholtz Zentrum Muenchen Deutsches Forschungszentrum fuer Gesundheit und Umwelt (GmbH). The sequence listing filed with the application follows.

SEQUENCE LISTING (5 sequences)

SEQ ID NO: 1 - RNA, 21 nt, Homo sapiens
ugguagacuauggaacguagg

SEQ ID NO: 2 - RNA, 25 nt, Homo sapiens
aagggauucugauguuggucacacu

SEQ ID NO: 3 - DNA, 15 bp, artificial sequence
  inhibitor of miR-379
gttccatagtctacc

SEQ ID NO: 4 - DNA, 16 bp, artificial sequence
  inhibitor of miR-541
caacatcagaatccct

SEQ ID NO: 5 - RNA, 122 nt, artificial sequence
  inhibitory sequence to miR-379 and miR-541 comprises by tough decoys
gacggcgcuaggaucaucaacagugugaccaacaucaucuagaaucccuucaaguauucuggucacagaauacaacccuacguuccaaucuuagucuaccacaagaugauccuagcgccguc